European Patent Application EP 4 249 599 A1, published September 27, 2023. Title: 一种CD7-CAR-T细胞的制备方法及应用. Applicant: 博生吉医药科技（苏州）有限公司 博生吉安科细胞技术有限公司. The sequence listing filed with the application follows.

SEQUENCE LISTING (20 sequences)

SEQ ID NO: 1 - DNA, 933 bp, 人工序列(Artificial Sequence)
atgctgctgctggtgacctctctgctgctctgcgaactgcctcacccagcctttctgctgatccccatggacgtgcagctgcaggaaagcggaggaggactggtgcaggcaggaggatctctgaggctgtcttgcgcagtgtccggatacccctacagcagctactgcatgggttggttcagacaggccccaggaaaggagagagagggagtggccgctatcgatagcgacggaagaaccagatacgccgacagcgtgaagggcaggttcaccatcagccaggacaacgccaagaacaccctgtacctgcagatgaaccggatgaagcccgaggacaccgccatgtactattgcgccgctcgcttcggacctatgggttgcgtggatctgagcaccctgagctttggccattggggacagggaacccaggtcaccgtgtccatcactggaggaggaggaagcggaggaggaggatctggaggaggaggaagcggaggaggaggatctatggacgtgcagctgcaggagagcggaggaggactggtgcaggcaggaggatctctgagactgtcttgcgccgtgtccggatacccttacagcagctactgcatgggctggttcaggcaggctccaggaaaggagagagagggagtggcagccatcgatagcgacggcagaaccagatacgccgatagcgtgaagggcaggttcaccatcagccaggacaacgccaagaacaccctgtacctgcagatgaaccggatgaagcccgaggataccgccatgtactattgcgccgccaggttcggacctatgggttgcgtggacctgagcacactgagcttcggccattggggacagggaacacaggtcaccgtgtccatcaccgagcagaagctgatcagcgaggaggacctgaaggacgagctgtga

SEQ ID NO: 2 - protein, 310 aa, 人工序列(Artificial Sequence)
MLLLVTSLLLCELPHPAFLLIPMDVQLQESGGGLVQAGGSLRLSCAVSGYPYSSYCMGWFRQAPGKEREGVAAIDSDGRTRYADSVKGRFTISQDNAKNTLYLQMNRMKPEDTAMYYCAARFGPMGCVDLSTLSFGHWGQGTQVTVSITGGGGSGGGGSGGGGSGGGGSMDVQLQESGGGLVQAGGSLRLSCAVSGYPYSSYCMGWFRQAPGKEREGVAAIDSDGRTRYADSVKGRFTISQDNAKNTLYLQMNRMKPEDTAMYYCAARFGPMGCVDLSTLSFGHWGQGTQVTVSITEQKLISEEDLKDEL

SEQ ID NO: 3 - DNA, 66 bp, 人工序列(Artificial Sequence)
atgctgctgctggtgacctctctgctgctctgcgaactgcctcacccagcctttctgctgatcccc

SEQ ID NO: 4 - protein, 22 aa, 人工序列(Artificial Sequence)
MLLLVTSLLLCELPHPAFLLIP

SEQ ID NO: 5 - DNA, 381 bp, 人工序列(Artificial Sequence)
atggacgtgcagctgcaggaaagcggaggaggactggtgcaggcaggaggatctctgaggctgtcttgcgcagtgtccggatacccctacagcagctactgcatgggttggttcagacaggccccaggaaaggagagagagggagtggccgctatcgatagcgacggaagaaccagatacgccgacagcgtgaagggcaggttcaccatcagccaggacaacgccaagaacaccctgtacctgcagatgaaccggatgaagcccgaggacaccgccatgtactattgcgccgctcgcttcggacctatgggttgcgtggatctgagcaccctgagctttggccattggggacagggaacccaggtcaccgtgtccatcact

SEQ ID NO: 6 - protein, 127 aa, 人工序列(Artificial Sequence)
MDVQLQESGGGLVQAGGSLRLSCAVSGYPYSSYCMGWFRQAPGKEREGVAAIDSDGRTRYADSVKGRFTISQDNAKNTLYLQMNRMKPEDTAMYYCAARFGPMGCVDLSTLSFGHWGQGTQVTVSIT

SEQ ID NO: 7 - DNA, 60 bp, 人工序列(Artificial Sequence)
ggaggaggaggaagcggaggaggaggatctggaggaggaggaagcggaggaggaggatct

SEQ ID NO: 8 - protein, 20 aa, 人工序列(Artificial Sequence)
GGGGSGGGGSGGGGSGGGGS

SEQ ID NO: 9 - DNA, 42 bp, 人工序列(Artificial Sequence)
gagcagaagctgatcagcgaggaggacctgaaggacgagctg

SEQ ID NO: 10 - protein, 14 aa, 人工序列(Artificial Sequence)
EQKLISEEDLKDEL

SEQ ID NO: 11 - DNA, 1770 bp, 人工序列(Artificial Sequence)
atgctgctgctggtgacctctctgctgctctgcgaactgcctcacccagcctttctgctgatccccatgcaggtgcagctggtggaaagcggaggaggactggtgcagccaggaggatctctgagactgtcttgcgccgccagcggctacccctacagcagctactgcatgggttggttcagacaggccccaggacagggactggaagcagtggcagccatcgatagcgacggcagaacacgctacgccgattccgtgaagggcagattcaccatcagccgggacaacagcaagaacaccctgtacctgcagatgaacagcctgagggccgaggataccgcagtgtactattgcgccgcccgctttggacctatgggttgcgtggacctgagcacactgagcttcggccattggggacagggaacactggtgacagtgtccagcgagagcaaatacggccctccttgccctccttgcccagccccagaatttgagggaggacctagcgtgttcctgttccctcccaagcccaaggacaccctgatgatcagccggaccccagaagtcacctgcgtggtggtggacgtgtctcaggaagaccccgaggtgcagttcaattggtacgtggacggcgtggaagtgcacaacgccaagaccaagcccagagaggagcagttccagagcacctacagagtggtgtccgtgctgaccgtgctgcatcaggattggctgaacggcaaggagtacaagtgcaaggtgtccaacaagggcctgcctagcagcatcgagaagaccatcagcaaggccaagggccagcctagagagcctcaggtgtacacactgcccccttctcaggaggagatgaccaagaaccaggtgtccctgacttgcctcgtgaagggcttctaccccagcgatattgccgtggagtgggagtctaacggccagcccgagaacaactacaagaccacccctcccgtgctggatagcgacggctctttcttcctgtacagccggctgacagtggacaaaagtcgctggcaggagggcaacgtgttcagttgcagcgtgatgcacgaggccctgcacaaccactacacccagaagagcctgtctctgtctctcggcaagtggctccctatcggttgcgccgcctttgtcgtcgtctgtatcctcggctgcatcctcatctgttggctcaccaagaagaagtacagcagcagcgtgcacgaccccaacggcgagtacatgttcatgcgggccgtcaacaccgccaagaagagcagactgaccgacgtgaccctgaagagaggcaggaagaagctgctgtacatcttcaagcagcccttcatgcggccagtgcagacaacccaggaggaagacggctgctcttgcagattccccgaggaagaagagggcggttgcgagctgagagtgaagttcagcagaagcgccgacgctccagcctatcagcagggccagaaccagctgtacaacgagctgaacctgggcaggagagaggagtacgacgtgctggacaagaggagaggcagagacccagagatgggcggcaagcctagacggaagaaccctcaggagggcctgtacaacgaactgcagaaggacaagatggccgaggcctacagcgagatcggcatgaagggcgagaggagaagaggcaagggacacgacggactgtaccagggactgagcacagccaccaaggacacatacgacgccctgcacatgcaggctctgcctcctagatga

SEQ ID NO: 12 - protein, 589 aa, 人工序列(Artificial Sequence)
MLLLVTSLLLCELPHPAFLLIPMQVQLVESGGGLVQPGGSLRLSCAASGYPYSSYCMGWFRQAPGQGLEAVAAIDSDGRTRYADSVKGRFTISRDNSKNTLYLQMNSLRAEDTAVYYCAARFGPMGCVDLSTLSFGHWGQGTLVTVSSESKYGPPCPPCPAPEFEGGPSVFLFPPKPKDTLMISRTPEVTCVVVDVSQEDPEVQFNWYVDGVEVHNAKTKPREEQFQSTYRVVSVLTVLHQDWLNGKEYKCKVSNKGLPSSIEKTISKAKGQPREPQVYTLPPSQEEMTKNQVSLTCLVKGFYPSDIAVEWESNGQPENNYKTTPPVLDSDGSFFLYSRLTVDKSRWQEGNVFSCSVMHEALHNHYTQKSLSLSLGKWLPIGCAAFVVVCILGCILICWLTKKKYSSSVHDPNGEYMFMRAVNTAKKSRLTDVTLKRGRKKLLYIFKQPFMRPVQTTQEEDGCSCRFPEEEEGGCELRVKFSRSADAPAYQQGQNQLYNELNLGRREEYDVLDKRRGRDPEMGGKPRRKNPQEGLYNELQKDKMAEAYSEIGMKGERRRGKGHDGLYQGLSTATKDTYDALHMQALPPR

SEQ ID NO: 13 - protein, 126 aa, 人工序列(Artificial Sequence)
MQVQLVESGGGLVQPGGSLRLSCAASGYPYSSYCMGWFRQAPGQGLEAVAAIDSDGRTRYADSVKGRFTISRDNSKNTLYLQMNSLRAEDTAVYYCAARFGPMGCVDLSTLSFGHWGQGTLVTVSS

SEQ ID NO: 14 - protein, 229 aa, 人工序列(Artificial Sequence)
ESKYGPPCPPCPAPEFEGGPSVFLFPPKPKDTLMISRTPEVTCVVVDVSQEDPEVQFNWYVDGVEVHNAKTKPREEQFQSTYRVVSVLTVLHQDWLNGKEYKCKVSNKGLPSSIEKTISKAKGQPREPQVYTLPPSQEEMTKNQVSLTCLVKGFYPSDIAVEWESNGQPENNYKTTPPVLDSDGSFFLYSRLTVDKSRWQEGNVFSCSVMHEALHNHYTQKSLSLSLGK

SEQ ID NO: 15 - protein, 23 aa, 人工序列(Artificial Sequence)
WLPIGCAAFVVVCILGCILICWL

SEQ ID NO: 16 - protein, 35 aa, 人工序列(Artificial Sequence)
TKKKYSSSVHDPNGEYMFMRAVNTAKKSRLTDVTL

SEQ ID NO: 17 - protein, 42 aa, 人工序列(Artificial Sequence)
KRGRKKLLYIFKQPFMRPVQTTQEEDGCSCRFPEEEEGGCEL

SEQ ID NO: 18 - protein, 112 aa, 人工序列(Artificial Sequence)
RVKFSRSADAPAYQQGQNQLYNELNLGRREEYDVLDKRRGRDPEMGGKPRRKNPQEGLYNELQKDKMAEAYSEIGMKGERRRGKGHDGLYQGLSTATKDTYDALHMQALPPR

SEQ ID NO: 19 - protein, 18 aa, 人工序列(Artificial Sequence)
EGRGSLLTCGDVEENPGP

SEQ ID NO: 20 - protein, 352 aa, 人工序列(Artificial Sequence)
MWLQSLLLLGTVACSISRKVCNGIGIGEFKDSLSINATNIKHFKNCTSISGDLHILPVAFRGDSFTHTPPLDPQELDILKTVKEITGFLLIQAWPENRTDLHAFENLEIIRGRTKQHGQFSLAVVSLNITSLGLRSLKEISDGDVIISGNKNLCYANTINWKKLFGTSGQKTKIISNRGENSCKATGQVCHALCSPEGCWGPEPRDCVSCRNVSRGRECVDKCNLLEGEPREFVENSECIQCHPECLPQAMNITCTGRGPDNCIQCAHYIDGPHCVKTCPAGVMGENNTLVWKYADAGHVCHLCHPNCTYGCTGPGLEGCPTNGPKIPSIATGMVGALLLLLVVALGIGLFM